European Patent Application EP 4 570 820 A1, published June 18, 2025. Title: 一种长效胰岛素化合物. Applicant: 成都奥达生物科技有限公司. Application CN. The sequence listing filed with the application follows.

SEQUENCE LISTING (12 sequences)

SEQ ID NO: 1 - protein, 21 aa, synthetic construct
  DISULFID 6..20: note = 6..11; note (original language) = 第6位半胱氨酸与第11位半胱氨酸通过链内二硫键连接
  SITE 7..20: note = 20; note (original language) = 第20位半胱氨酸与SEQ ID NO.2或SEQ ID NO.3所示的第19位半胱氨酸通过链间二硫键连接; note = 7; note (original language) = 第7位半胱氨酸与SEQ ID NO.2或SEQ ID NO.3所示的第7位半胱氨酸通过链间二硫键连接
GIVEQCCTSICSLEQLENYCN

SEQ ID NO: 2 - protein, 29 aa, synthetic construct
  SITE 7..19: note = 7; note (original language) = 第7位半胱氨酸与SEQ ID NO.1所示的第7位半胱氨酸通过链间二硫键连接; note = 19; note (original language) = 第19位半胱氨酸与SEQ ID NO.1所示的第20位半胱氨酸通过链间二硫键连接
  MOD_RES 29: note = 29; note (original language) = 为PEG5CH2CO-γGlu-二十烷二酸修饰的赖氨酸
FVNQHLCGSHLVEALELVCGERGFHYTPX

SEQ ID NO: 3 - protein, 31 aa, synthetic construct
  SITE 7..19: note = 7; note (original language) = 第7位半胱氨酸与SEQ ID NO.1所示的第7位半胱氨酸通过链间二硫键连接; note = 19; note (original language) = 第19位半胱氨酸与SEQ ID NO.1所示的半胱氨酸通过链间二硫键连接
  MOD_RES 31: note = 31; note (original language) = 为PEG5CH2CO-γGlu-二十烷二酸修饰的赖氨酸
FVNQHLCGSHLVEALELVCGERGFHYTPKTX

SEQ ID NO: 4 - protein, 21 aa, synthetic construct
  DISULFID 6..11: note = 6..11; note (original language) = 第6位半胱氨酸与第11位半胱氨酸由链内二硫键连接
  SITE 7..20: note = 7; note (original language) = 第7位半胱氨酸与SEQ ID NO.5或SEQ ID NO.6所示的第7位半胱氨酸通过链间二硫键连接; note = 20; note (original language) = 第20位天冬氨酸与SEQ ID NO.5或SEQ ID NO.6所示的第19位X连接
GIVEQCCTSICSLEQLENYDN

SEQ ID NO: 5 - protein, 29 aa, synthetic construct
  MOD_RES 19..29: note = 29; note (original language) = X为PEG5CH2CO-γGlu-二十烷二酸修饰的赖氨酸; note = 19; note (original language) = X为Dap
  SITE 7..19: note = 7; note (original language) = 第7位半胱氨酸与SEQ ID NO.4所示的第7位半胱氨酸通过链间二硫键连接; note = 19; note (original language) = 第19位X与SEQ ID NO.4所示的天冬氨酸连接
FVNQHLCGSHLVEALELVXGERGFHYTPX

SEQ ID NO: 6 - protein, 31 aa
FVNQHLCGSHLVEALELVXGERGFHYTPKTX

SEQ ID NO: 7 - protein, 21 aa, synthetic construct
  MOD_RES 20: note = 20; note (original language) = X为L-4-溴-2-氨基丁酰胺
  DISULFID 6..11: note = 6..11; note (original language) = 第6位半胱氨酸与第11位半胱氨酸由链内二硫键连接
  SITE 7..20: note = 7; note (original language) = 第7位半胱氨酸与SEQ ID NO.8或SEQ ID NO.9所示的第7位半胱氨酸通过链间二硫键连接; note = 20; note (original language) = 第20位X与SEQ ID NO.8或SEQ ID NO.9所示的第19位半胱氨酸连接
GIVEQCCTSICSLEQLENYXN

SEQ ID NO: 8 - protein, 29 aa, synthetic construct
  MOD_RES 29: note = 29; note (original language) = X为PEG5CH2CO-γGlu-二十烷二酸修饰的赖氨酸
  SITE 7..19: note = 7; note (original language) = 第7为半胱氨酸与SEQ ID NO.7所示的第7为半胱氨酸通过链间二硫键连接; note = 20; note (original language) = 第19位半胱氨酸与SEQ ID NO.7所示的第20位X连接
FVNQHLCGSHLVEALELVCGERGFHYTPX

SEQ ID NO: 9 - protein, 31 aa, synthetic construct; identical to SEQ ID NO: 3
  MOD_RES 31: note = 31; note (original language) = X为PEG5CH2CO-γGlu-二十烷二酸修饰的赖氨酸
  SITE 7..19: note = 19; note (original language) = 第19位的半胱氨酸与SEQ ID NO.7所示的第20位X连接; note = 7; note (original language) = 第7位半胱氨酸与SEQ ID NO.7所示的第7位半胱氨酸通过链间二硫键连接

SEQ ID NO: 10 - protein, 19 aa
GIVEQCCTSICSLEQLENY

SEQ ID NO: 11 - protein, 29 aa, synthetic construct
  MOD_RES 19..29: note = 29; note (original language) = X为PEG5CH2CO-γGlu-二十烷二酸修饰的赖氨酸; note = 19; note (original language) = X为(S,S) DAS[Dde-Asn(Trt)-OtBu]
  SITE 7..19: note = 19; note (original language) = 第19位X与SEQ ID NO.10所示的第19位酪氨酸连接; note = 7; note (original language) = 第7位半胱氨酸与SEQ ID NO.10所示的第7位半胱氨酸通过链间二硫键连接
FVNQHLCGSHLVEALELVXGERGFHYTPX

SEQ ID NO: 12 - protein, 31 aa, synthetic construct; identical to SEQ ID NO: 6
  MOD_RES 19..31: note = 31; note (original language) = X为PEG5CH2CO-γGlu-二十烷二酸修饰的赖氨酸; note = 19; note (original language) = X为(S,S) DAS[Dde-Asn(Trt)-OtBu]
  SITE 7..19: note = 7; note (original language) = 第7位半胱氨酸与SEQ ID NO.10所示的第7位半胱氨酸通过链间二硫键连接; note = 19; note (original language) = 第19位X与SEQ ID NO.10所示的第19位酪氨酸连接